European Patent Specification EP 3 836 949 B1, published June 24, 2026. Title: COMPOSITIONS COMPRISING SEL1-DERIVED PEPTIDES AND METHODS OF TREATMENT/PREVENTION OF EXCESS OXALATE LEVELS AND ASSOCIATED CONDITIONS/DISEASES THEREWITH. Applicant: The University of Chicago. The sequence listing filed with the application follows.

SEQUENCE LISTING (47 sequences)

SEQ ID NO: 1 - DNA, 1572 bp, Artificial sequence
  Synthetic
atgtcgtccgtcattgctgattcgcagcagcctgcagtttcagaagaaaacgcaaataaaattatccttgatgaggaaaaggcggtcatccaatgtaacgaaagatataagacggaaaatgatgaaaagggcgatgaagaaaccgtttcatggtgccgaaaagccgcgaagtctggtaatgcggaggcacaatatctttttggcatgctggtttatgatggcagaggcgtgcagcaggataattgtgttgccatgttatggtggatgaaagcagcagagcagaatcatgccaaggcactcgttatgctgggaaatcttcatcgtaaaggtcagtgcattgctgagaattatccgaaagccattgcctattggaagagagctgctgttcagaataacgtatgggcatatcataatttagggacagcttattacgatggtatcggtgtggataaaaatcctcatgaagctgttcgctggtggaagaaggcagccgaattgggttttcctgaatctcagaacaatctgggtgctttatacaatgatgggaatggtgttgatcgtgattatcaggaggctgttttctggtacagaaaaagtgccctgcagggcgacgaattgggacagtacaatcttggggtggcttattattacggcagagggataaaaaaagatttttctgaagcagtgtcgtggtacaaaaaatcagcagaacaagactatgcacaagcacagcataatcttggtgttacgtattacgaaggtgagggaataaaaaaagattacgccaaggctgtgtactggtggaaaaaggcagcagaacaggggattccccaatctcagtataaccttggcattgcatatgaagaaggctggggcgctgaaaaaaatccggagaatgctgttttttggtacagaaaagcggctgaacagggacatgctgatgctcaaaacagacttggcatcgcttacaggtatggaaccggagtcaggaaaaatcccgcattgtctgtcaaatggctggaaaaagcggcaaagcaggggcttgcaagagcacagttcaatttggggaaaaccttctatatcggagcaggcattaacaagaatacagacaaagcggtttactggttcataaaagctgccaatcagggtttcacagaagcacaggcttatattggtatgatttattttaaaggtaaatatgtcgccaagaacgaaaaaaaaggtttttactggttaaaaaaagcagcagaaaaagacagtgctaaagcacaagcatttcttggcgctttatacattgcaggaaatgaagtgaagccaaatataaaggaaggcgttgccttgacaaaaaaagcggcattacagggtaattacgaggcacaaaccctgctcggtttttgctacgagaatggcttggaagtaaaaaaagacctgattgccgcatatgcgctttacttgtcggcgtcacctcatttcgattttgcagaaaaggcgcgtcttgatcttgaacggaaattaagcgaacaggaaatagcaaaggcaatatccgttaatacagcaaaattgtttgagtga

SEQ ID NO: 2 - protein, 523 aa, Artificial sequence
  Synthetic
MSSVIADSQQPAVSEENANKIILDEEKAVIQCNERYKTENDEKGDEETVSWCRKAAKSGNAEAQYLFGMLVYDGRGVQQDNCVAMLWWMKAAEQNHAKALVMLGNLHRKGQCIAENYPKAIAYWKRAAVQNNVWAYHNLGTAYYDGIGVDKNPHEAVRWWKKAAELGFPESQNNLGALYNDGNGVDRDYQEAVFWYRKSALQGDELGQYNLGVAYYYGRGIKKDFSEAVSWYKKSAEQDYAQAQHNLGVTYYEGEGIKKDYAKAVYWWKKAAEQGIPQSQYNLGIAYEEGWGAEKNPENAVFWYRKAAEQGHADAQNRLGIAYRYGTGVRKNPALSVKWLEKAAKQGLARAQFNLGKTFYIGAGINKNTDKAVYWFIKAANQGFTEAQAYIGMIYFKGKYVAKNEKKGFYWLKKAAEKDSAKAQAFLGALYIAGNEVKPNIKEGVALTKKAALQGNYEAQTLLGFCYENGLEVKKDLIAAYALYLSASPHFDFAEKARLDLERKLSEQEIAKAISVNTAKLFE

SEQ ID NO: 3 - DNA, 1470 bp, Artificial sequence
  Synthetic
atgaaaagacgggttttgtatggtgtgctgtttgcggtgctggcggggtgttctgccggtgcgttggcgtccgtgtccggcttgtcggatgggctggcgcagcttgaacggaggcagttcgaatcggcttatgcgacgctcatgccggaggcggagaaggggaatccccgtgcggcgctggaggtggggaagctgctgttgacggggcgcggggtggcaaaggatgaagcggcggcggtgaagtggcttctggtggcggcggatagtggcaaccgggatgcgcagtatatgctgggggcgatgtcggtggaggggatcggtctgccgaaggattctcaggtggcgttgacctggctgtcgaaggcggcggcgcagggggatgcgcgtgcgaagacggctttggggattctgatgcagtccgccgggccgggatcgcagcatacggaacaggcagcccggtggttcgagagggcggcggcgtcaggggaaccggaggcgcaacggcgctgggcgctgatgctggcgtctggccggggggtggccaaaaatgagggtgaggcactgaaatggtttaagaaggcggctgtcgcgggggatgtggaagcgcagcgcaatctggggattatgctctcgacgggaaagggggtgacgggcggcaagccggattttgcggaagcggcacgctggtacggcctggcagcgaagaagggggatgcgaaggcgcagtatgggttgggcattttgtatgcgaaggggcagggggtggcgcccgatcaggaaaaggcgctgattctgtatcgcatggcggcgactcaggggctggcgacggcggagtatgccgtcgggctggcgtatgcgtatggacgggggacggcacaaaatgatgtgaaggcggccgactggttcgaggcggcggcgcagcagggggtggtgcgtgcgcaatataatctcgctctgatgctggaggcgggtcgcggtcggcctgtggatacggtggcggcgagcaagtggtttttgatggcggcggagaagggcttgcgggaggcacaatacaatatggggtatcactatgccgaggggaaaggggtgccacgcgatcagggcaaggcggtgttctggtatgaaaaggcggcggctgccggggatgtgaaggcccagtacaatctggggatgctgtatctgaacggggttaatggcaaggcggatgacgaaaaggcggcttttttctaccggatggcggccggggcgggatatggcccggcgatgtaccggctggcggtgttgtatgaggaaggccgtggggtaaagcagagttatcagctggcaggggaatggtatgagcgggcggatctggccgcgaaagtgaagattgacgaggcgatgaaaaagaatccgcatccgtttgtgcaacggactctgcaggtgccggatgatttgaatcaatcttcagataaattggcgggacattag

SEQ ID NO: 4 - protein, 489 aa, Artificial sequence
  Synthetic
MKRRVLYGVLFAVLAGCSAGALASVSGLSDGLAQLERRQFESAYATLMPEAEKGNPRAALEVGKLLLTGRGVAKDEAAAVKWLLVAADSGNRDAQYMLGAMSVEGIGLPKDSQVALTWLSKAAAQGDARAKTALGILMQSAGPGSQHTEQAARWFERAAASGEPEAQRRWALMLASGRGVAKNEGEALKWFKKAAVAGDVEAQRNLGIMLSTGKGVTGGKPDFAEAARWYGLAAKKGDAKAQYGLGILYAKGQGVAPDQEKALILYRMAATQGLATAEYAVGLAYAYGRGTAQNDVKAADWFEAAAQQGVVRAQYNLALMLEAGRGRPVDTVAASKWFLMAAEKGLREAQYNMGYHYAEGKGVPRDQGKAVFWYEKAAAAGDVKAQYNLGMLYLNGVNGKADDEKAAFFYRMAAGAGYGPAMYRLAVLYEEGRGVKQSYQLAGEWYERADLAAKVKIDEAMKKNPHPFVQRTLQVPDDLNQSSDKLAGH

SEQ ID NO: 5 - protein, 35 aa, Artificial sequence
  Synthetic
ADAQNRLGIAYRYGTGVRKNPALSVKWLEKAAKQG

SEQ ID NO: 6 - protein, 30 aa, Artificial sequence
  Synthetic
QYNLGVAYYYGRGIKKDFSEAVSWYKKSAE

SEQ ID NO: 7 - protein, 33 aa, Artificial sequence
  Synthetic
AYHNLGTAYYDGIGVDKNPHEAVRWWKKAAELG

SEQ ID NO: 8 - protein, 35 aa, Artificial sequence
  Synthetic
QSQYNLGIAYEEGWGAEKNPENAVFWYRKAAEQGH

SEQ ID NO: 9 - protein, 35 aa, Artificial sequence
  Synthetic
ARAQFNLGKTFYIGAGINKNTDKAVYWFIKAANQG

SEQ ID NO: 10 - protein, 35 aa, Artificial sequence
  Synthetic
ESQNNLGALYNDGNGVDRDYQEAVFWYRKSALQGD

SEQ ID NO: 11 - protein, 35 aa, Artificial sequence
  Synthetic
EAQYNMGYHYAEGKGVPRDQGKAVFWYEKAAAAGD

SEQ ID NO: 12 - protein, 35 aa, Artificial sequence
  Synthetic
DAQYMLGAMSVEGIGLPKDSQVALTWLSKAAAQGD

SEQ ID NO: 13 - protein, 35 aa, Artificial sequence
  Synthetic
AKAQYGLGILYAKGQGVAPDQEKALILYRMAATQG

SEQ ID NO: 14 - protein, 35 aa, Artificial sequence
  Synthetic
ATAEYAVGLAYAYGRGTAQNDVKAADWFEAAAQQG

SEQ ID NO: 15 - protein, 35 aa, Artificial sequence
  Synthetic
EAQRRWALMLASGRGVAKNEGEALKWFKKAAVAGD

SEQ ID NO: 16 - protein, 36 aa, Artificial sequence
  Synthetic
ALAQSNLGVLYASGRGVESSPKRALEWYKKAAVQGN

SEQ ID NO: 17 - protein, 36 aa, Artificial sequence
  Synthetic
SQAQFSLGNMYEDGSGVEKNLAVAAAWYQKSAEQGN

SEQ ID NO: 18 - protein, 28 aa, Artificial sequence
  Synthetic
AEAQTNLGVLYSYGLGVDKDLSKAFYWY

SEQ ID NO: 19 - protein, 34 aa, Artificial sequence
  Synthetic
ESQDRLGLMLTNGVGVKQDYKQAYSWFRKAARQG

SEQ ID NO: 20 - protein, 31 aa, Artificial sequence
  Synthetic
AESQNNLGVLYARGLGVEKDYKQAVAWYRKA

SEQ ID NO: 21 - protein, 33 aa, Artificial sequence
  Synthetic
QAQFNLGTMYLQGHGVKQDVKQARHWFTKAAAQ

SEQ ID NO: 22 - protein, 35 aa, Artificial sequence
  Synthetic
AQAQHNLGVTYYEGEGIKKDYAKAVYWWKKAAEQG

SEQ ID NO: 23 - protein, 36 aa, Artificial sequence
  Synthetic
PQSQYNLGIAYEEGWGAEKNPENAVFWYRKAAEQGH

SEQ ID NO: 24 - protein, 35 aa, Artificial sequence
  Synthetic
EAQAYIGMIYFKGKYVAKNEKKGFYWLKKAAEKDS

SEQ ID NO: 25 - protein, 33 aa, Artificial sequence
  Synthetic
ALYGLGVMATNGLGMPRNDEKALVWFREGAAKG

SEQ ID NO: 26 - protein, 34 aa, Artificial sequence
  Synthetic
EAQFGLGAMYDLSRGVRQDMTLAIDWYEKSARAG

SEQ ID NO: 27 - protein, 32 aa, Artificial sequence
  Synthetic
QLYLGLMYGHGKGVPRDLNKSLFWVEKAADRG

SEQ ID NO: 28 - protein, 34 aa, Artificial sequence
  Synthetic
AQYLMGMAYLEGKSVPQDLPVAAAWFYKAAMQGN

SEQ ID NO: 29 - protein, 36 aa, Artificial sequence
  Synthetic
ADAQLRLGYMYARGIGVPVDKPKAVAWLEKAASAGN

SEQ ID NO: 30 - protein, 29 aa, Artificial sequence
  Synthetic
GSMLSQGKGVEKDPKKGLEWFVQAGQDGD

SEQ ID NO: 31 - protein, 36 aa, Artificial sequence
  Synthetic
SEAQQMMGFLYGEGWGAKRDPVKAEYWFDKAAASGD

SEQ ID NO: 32 - protein, 34 aa, Artificial sequence
  Synthetic
QAEHEMGSLYLMGIGVAQSNVMAVAWYRKAAIQG

SEQ ID NO: 33 - protein, 36 aa, Artificial sequence
  Synthetic
APSQTAMGYAYEEGAGVPQDADLARYWFDKAAAQGN

SEQ ID NO: 34 - protein, 33 aa, Artificial sequence
  Synthetic
AQAGLGWMYAAGRGVNKDETLSFSWYERAAVAG

SEQ ID NO: 35 - protein, 34 aa, Artificial sequence
  Synthetic
AQYMLGRYYEKGIGVAKDRVLAKEWYEKAAAQGN

SEQ ID NO: 36 - protein, 80 aa, Artificial sequence
  Synthetic
KAAKSGNAEAQYLFGMLVYDGRGVQQDNCVAMLWWMKAAEQNHAKALVMLGNLHRKGQCIAENYPKAIAYWKRAAVQNNV

SEQ ID NO: 37 - protein, 98 aa, Artificial sequence
  Synthetic
LGTAYYDGIGVDKNPHEAVRWWKKAAELGFPESQNNLGALYNDGNGVDRDYQEAVFWYRKSALQGDELGQYNLGVAYYGRGIKKDFSEAVSWYKKSAE

SEQ ID NO: 38 - protein, 87 aa, Artificial sequence
  Synthetic
YRKAAEQGHADAQNRLGIAYRYGTGVRKNPALSVKWLEKAAKQGLARAQFNLGKTFYIGAGINKNTDKAVYWFIKAANQGFTEAQAY

SEQ ID NO: 39 - protein, 35 aa, Artificial sequence; identical to SEQ ID NO: 12
  Synthetic

SEQ ID NO: 40 - protein, 34 aa, Artificial sequence
  Synthetic
DAQYMLGAMSVEGILPKDSQVALTWLSKAAAQGD

SEQ ID NO: 41 - protein, 35 aa, Artificial sequence; identical to SEQ ID NO: 12
  Synthetic

SEQ ID NO: 42 - protein, 31 aa, Artificial sequence
  Synthetic
DAQYMLAMSVEILPKDSQVALTWLSKAAAQD

SEQ ID NO: 43 - protein, 35 aa, Artificial sequence; identical to SEQ ID NO: 13
  Synthetic

SEQ ID NO: 44 - protein, 34 aa, Artificial sequence
  Synthetic
AKAQYGLGILYAKGQVAPDQEKALILYRMAATQG

SEQ ID NO: 45 - protein, 35 aa, Artificial sequence; identical to SEQ ID NO: 13
  Synthetic

SEQ ID NO: 46 - protein, 30 aa, Artificial sequence
  Synthetic
AKAQYLILYAKQVAPDQEKALILYRMAATQ

SEQ ID NO: 47 - protein, 36 aa, Artificial sequence
  Synthetic
RDAQYMLGAMSVEGIGLPKDSQVALTWLSKAAAQGD